European Patent Application EP 4 745 241 A1, published May 20, 2026. Title: 一种用于过敏性疾病的基因治疗载体核酸构建体及其使用方法. Applicant: 康霖生物科技(杭州)有限公司. Application CN, filed July 2, 2024. The sequence listing filed with the application follows.

SEQUENCE LISTING (39 sequences)

SEQ ID NO: 1 - DNA, 4791 bp, synthetic construct
  source 1..4791: mol_type = other DNA
acatgtgagcaaaaggccagcaaaaggccaggaaccgtaaaaaggccgcgttgctggcgtttttccataggctccgcccccctgacgagcatcacaaaaatcgacgctcaagtcagaggtggcgaaacccgacaggactataaagataccaggcgtttccccctggaagctccctcgtgcgctctcctgttccgaccctgccgcttaccggatacctgtccgcctttctcccttcgggaagcgtggcgctttctcatagctcacgctgtaggtatctcagttcggtgtaggtcgttcgctccaagctgggctgtgtgcacgaaccccccgttcagcccgaccgctgcgccttatccggtaactatcgtcttgagtccaacccggtaagacacgacttatcgccactggcagcagccactggtaacaggattagcagagcgaggtatgtaggcggtgctacagagttcttgaagtggtggcctaactacggctacactagaaggacagtatttggtatctgcgctctgctgaagccagttaccttcggaaaaagagttggtagctcttgatccggcaaacaaaccaccgctggtagcggtggtttttttgtttgcaagcagcagattacgcgcagaaaaaaaggatctcaagaagatcctttgatcttttctacggggtctgacgctcagtggaacgaaaactcacgttaagggattttggtcatgagattatcaaaaaggatcttcacctagatccttttaaattaaaaatgaagttttaaatcaatctaaagtatatatgagtaaacttggtctgacagttaccaatgcttaatcagtgaggcacctatctcagcgatctgtctatttcgttcatccatagttgcctgactccccgtcgtgtagataactacgatacgggagggcttaccatctggccccagtgctgcaatgataccgcgagacccacgctcaccggctccagatttatcagcaataaaccagccagccggaagggccgagcgcagaagtggtcctgcaactttatccgcctccatccagtctattaattgttgccgggaagctagagtaagtagttcgccagttaatagtttgcgcaacgttgttgccattgctacaggcatcgtggtgtcacgctcgtcgtttggtatggcttcattcagctccggttcccaacgatcaaggcgagttacatgatcccccatgttgtgcaaaaaagcggttagctccttcggtcctccgatcgttgtcagaagtaagttggccgcagtgttatcactcatggttatggcagcactgcataattctcttactgtcatgccatccgtaagatgcttttctgtgactggtgagtactcaaccaagtcattctgagaatagtgtatgcggcgaccgagttgctcttgcccggcgtcaatacgggataataccgcgccacatagcagaactttaaaagtgctcatcattggaaaacgttcttcggggcgaaaactctcaaggatcttaccgctgttgagatccagttcgatgtaacccactcgtgcacccaactgatcttcagcatcttttactttcaccagcgtttctgggtgagcaaaaacaggaaggcaaaatgccgcaaaaaagggaataagggcgacacggaaatgttgaatactcatactcttcctttttcaatattattgaagcatttatcagggttattgtctcatgagcggatacatatttgaatgtatttagaaaaataaacaaataggggttccgcgcacatttccccgaaaagtgccacctgacgtctaagaaaccattattatcatgacattaacctataaaaataggcgtatcacgaggccctttcgtctcgcgcgtttcggtgatgacggtgaaaacctctgacacatgcagctcccggagacggtcacagcttgtctgtaagcggatgccgggagcagacaagcccgtcagggcgcgtcagcgggtgttggcgggtgtcggggctggcttaactatgcggcatcagagcagattgtactgagagtgcaccataaaattgtaaacgttaatattttgttaaaattcgcgttaaatttttgttaaatcagctcattttttaaccaataggccgaaatcggcaaaatcccttataaatcaaaagaatagcccgagatagggttgagtgttgttccagtttggaacaagagtccactattaaagaacgtggactccaacgtcaaagggcgaaaaaccgtctatcagggcgatggcccactacgtgaaccatcacccaaatcaagttttttggggtcgaggtgccgtaaagcactaaatcggaaccctaaagggagcccccgatttagagcttgacggggaaagccggcgaacgtggcgagaaaggaagggaagaaagcgaaaggagcgggcgctagggcgctggcaagtgtagcggtcacgctgcgcgtaaccaccacacccgccgcgcttaatgcgccgctacagggcgcgtactatggttgctttgacgtatgcggtgtgaaataccgcacagatgcgtaaggagaaaataccgcatcaggcgcccctgcaggcagctgcgcgctcgctcgctcactgaggccgcccgggcaaagcccgggcgtcgggcgacctttggtcgcccggcctcagtgagcgagcgagcgcgcagagagggagtggccaactccatcactaggggttcctacgcgtcgttacataacttacggtaaatggcccgcctggctgaccgcccaacgacccccgcccattgacgtcaataatgacgtatgttcccatagtaacgccaatagggactttccattgacgtcaatgggtggagtatttacggtaaactgcccacttggcagtacatcaagtgtatcatatgccaagtacgccccctattgacgtcaatgacggtaaatggcccgcctggcattatgcccagtacatgaccttatgggactttcctacttggcagtacatctacgtattagtcatcgctattaccatggtcgaggtgagccccacgttctgcttcactctccccatctcccccccctccccacccccaattttgtatttatttattttttaattattttgtgcagcgatgggggcggggggggggggggggcgcgcgccaggcggggcggggcggggcgaggggcggggcggggcgaggcggagaggtgcggcggcagccaatcagagcggcgcgctccgaaagtttccttttatggcgaggcggcggcggcggcggccctataaaaagcgaagcgcgcggcgggcgggagtcgctgcgacgctgccttcgccccgtgccccgctccgccgccgcctcgcgccgcccgccccggctctgactgaccgcgttactcccacaggtgagcgggcgggacggcccttctcctccgggctgtaattagctgagcaagaggtaagggtttaagggatggttggttggtggggtattaatgtttaattacctggagcacctgcctgaaatcactttttttcaggttggaccggtgccaccatggccctccttacgaacctcctgccgttgtgctgcctggccctcctcgccttgccagcgcagagccacgccgaaggcacgttcacctccgacgtgagcagctacctggagggccaggccgcgaaagagttcatcgcttggctcgtcaagggcggaggaggaggcggaggaagcggcggaggaggaagcggaggcggaggtagcgccgagagcaagtacggccctccttgtcctccctgccctgccccagaggccgctggaggaccatccgtgtttctgtttccccccaagcctaaggacaccctgatgatcagcaggacccccgaggtgacctgcgtggtggtggacgtgagccaggaggaccctgaggtgcagttcaattggtacgtggatggcgtggaggtgcacaacgccaagacaaagcccagagaggagcagtttaatagcacctacagagtggtgtccgtgctgaccgtgctgcaccaggattggctgaatggcaaggagtacaagtgcaaggtgtccaataagggcctgcccagcagcatcgagaagaccatcagcaaggccaagggccagcccagagagcctcaggtgtacacactgcctccctcccaggaggagatgaccaagaaccaggtgtccctgacctgtctggtgaagggcttctaccccagcgatatcgccgtggagtgggagtccaacggccagcccgagaataactacaagaccacccctcctgtgctggatagcgacggcagctttttcctgtactccagactgaccgtggacaagtctagatggcaggagggcaacgtgttttcttgtagcgtgatgcacgaggccctgcacaatcactacacccagaagtccctgtctctgagcctgggctgagtcgacgtttatttgtgaaatttgtgatgctattgctttatttgtaaccatctagctttatttgtgaaatttgtgatgctattgctttatttgtaaccattataagctgcaataaacaagttaacaacaacaattgcattcattttatgtttcaggttcagggggagatgtgggaggttttttaaagtttaaacaggaacccctagtgatggagttggccactccctctctgcgcgctcgctcgctcactgaggccgggcgaccaaaggtcgcccgacgcccgggcggcctcagtgagcgagcgagcgcgcagctgcctgcagg

SEQ ID NO: 2 - DNA, 24 bp, synthetic construct
  source 1..24: mol_type = other DNA
ggatagcaaggacagcacatactc

SEQ ID NO: 3 - DNA, 20 bp, synthetic construct
  source 1..20: mol_type = other DNA
gtgagctatgagaaagcgcc

SEQ ID NO: 4 - DNA, 814 bp, synthetic construct
  source 1..814: mol_type = other DNA
cgttacataacttacggtaaatggcccgcctggctgaccgcccaacgacccccgcccattgacgtcaataatgacgtatgttcccatagtaacgccaatagggactttccattgacgtcaatgggtggagtatttacggtaaactgcccacttggcagtacatcaagtgtatcatatgccaagtacgccccctattgacgtcaatgacggtaaatggcccgcctggcattatgcccagtacatgaccttatgggactttcctacttggcagtacatctacgtattagtcatcgctattaccatggtcgaggtgagccccacgttctgcttcactctccccatctcccccccctccccacccccaattttgtatttatttattttttaattattttgtgcagcgatgggggcggggggggggggggggcgcgcgccaggcggggcggggcggggcgaggggcggggcggggcgaggcggagaggtgcggcggcagccaatcagagcggcgcgctccgaaagtttccttttatggcgaggcggcggcggcggcggccctataaaaagcgaagcgcgcggcgggcgggagtcgctgcgacgctgccttcgccccgtgccccgctccgccgccgcctcgcgccgcccgccccggctctgactgaccgcgttactcccacaggtgagcgggcgggacggcccttctcctccgggctgtaattagctgagcaagaggtaagggtttaagggatggttggttggtggggtattaatgtttaattacctggagcacctgcctgaaatcactttttttcaggt

SEQ ID NO: 5 - DNA, 1359 bp, synthetic construct
  source 1..1359: mol_type = other DNA
caggtgcagctggtgcagtccggcgctgaggtcatgaagcccggcagctccgtgaaggtgtcctgcaaggcctccggctacacctttagctggtactggctggagtgggtgaggcaggcccctggccacggactggagtggatgggcgagatcgaccctggcacattcactacaaactacaacgagaagttcaaggccagggtgaccttcacagccgatacaagcacctccacagcctacatggagctgagcagcctgaggtccgaggacaccgccgtgtactactgtgccagattttcccacttcagcggctccaactacgactactttgattactggggccagggcacactggtgaccgtgagcagcgcctccaccaagggcccttccgtgttccctctggcccctagctccaagtccacctccggcggcaccgccgctctgggatgtctggtgaaggactacttccccgagcctgtgaccgtgtcctggaactccggcgccctgacatccggcgtgcacaccttccccgccgtgctgcagagctccggcctgtactccctgagcagcgtggtgacagtgccttccagctccctgggcacacagacctacatctgcaacgtgaaccacaagccttccaataccaaggtggacaagaaggtggagcccaagagctgtgataagacccacacctgtcccccttgccctgcccccgagctgctgggaggaccatccgtgttcctgttccctcctaagcctaaggacaccctgatgatctccaggacccccgaggtgacctgcgtggtggtggacgtgtcccacgaggaccctgaggtgaagttcaactggtacgtggatggcgtggaggtgcacaacgccaagacaaagcctagggaggagcagtacaatagcacatacagagtggtgagcgtgctgaccgtgctgcaccaggactggctgaatggcaaggagtacaagtgtaaggtgagcaataaggccctgcccgcccccatcgagaagacaatctccaaggccaagggccagcctagagagccccaggtgtacacactgcccccctccagagacgagctgacaaagaaccaggtgtccctgacatgtctggtgaaaggcttttaccccagcgatatcgccgtggagtgggagagcaatggccagcccgagaataattacaagaccacccctcccgtgctggactccgatggcagctttttcctgtacagcaagctgaccgtggacaagagcagatggcagcagggcaacgtgttctcctgctccgtgatgcacgaggccctgcacaaccactacacccagaagtccctgtccctgtcccctggcaag

SEQ ID NO: 6 - protein, 453 aa, synthetic construct
QVQLVQSGAEVMKPGSSVKVSCKASGYTFSWYWLEWVRQAPGHGLEWMGEIDPGTFTTNYNEKFKARVTFTADTSTSTAYMELSSLRSEDTAVYYCARFSHFSGSNYDYFDYWGQGTLVTVSSASTKGPSVFPLAPSSKSTSGGTAALGCLVKDYFPEPVTVSWNSGALTSGVHTFPAVLQSSGLYSLSSVVTVPSSSLGTQTYICNVNHKPSNTKVDKKVEPKSCDKTHTCPPCPAPELLGGPSVFLFPPKPKDTLMISRTPEVTCVVVDVSHEDPEVKFNWYVDGVEVHNAKTKPREEQYNSTYRVVSVLTVLHQDWLNGKEYKCKVSNKALPAPIEKTISKAKGQPREPQVYTLPPSRDELTKNQVSLTCLVKGFYPSDIAVEWESNGQPENNYKTTPPVLDSDGSFFLYSKLTVDKSRWQQGNVFSCSVMHEALHNHYTQKSLSLSPGK

SEQ ID NO: 7 - DNA, 642 bp, synthetic construct
  source 1..642: mol_type = other DNA
gagatcgtgatgacacagtcccccgccaccctgtccgtgagcccaggagagagggccacactgagctgcagggcctcccagagcatcggcaccaatatccactggtaccagcagaagcccggccaggcccctaggctgctgatctactacgcctccgagtccatcagcggcatccccgccagattcagcggcagcggcagcggaaccgagtttaccctgacaatctcctccctgcagtccgaggacttcgccgtgtactattgtcagcagagctggtcctggcccaccacctttggcggcggcacaaaggtggagatcaagaggacagtggccgcccctagcgtgtttatcttcccccccagcgacgagcagctgaagtccggcaccgccagcgtggtgtgtctgctgaacaacttttaccctagggaggccaaggtgcagtggaaggtggataatgccctgcagagcggcaattcccaggagtccgtgacagagcaggatagcaaggacagcacatactccctgtccagcaccctgacactgtccaaggccgactacgagaagcacaaggtgtacgcctgcgaggtgacacaccagggcctgtcctcccctgtgacaaagagcttcaacagaggcgagtgc

SEQ ID NO: 8 - protein, 214 aa, synthetic construct
EIVMTQSPATLSVSPGERATLSCRASQSIGTNIHWYQQKPGQAPRLLIYYASESISGIPARFSGSGSGTEFTLTISSLQSEDFAVYYCQQSWSWPTTFGGGTKVEIKRTVAAPSVFIFPPSDEQLKSGTASVVCLLNNFYPREAKVQWKVDNALQSGNSQESVTEQDSKDSTYSLSSTLTLSKADYEKHKVYACEVTHQGLSSPVTKSFNRGEC

SEQ ID NO: 9 - DNA, 180 bp, synthetic construct
  source 1..180: mol_type = other DNA
gtttatttgtgaaatttgtgatgctattgctttatttgtaaccatctagctttatttgtgaaatttgtgatgctattgctttatttgtaaccattataagctgcaataaacaagttaacaacaacaattgcattcattttatgtttcaggttcagggggagatgtgggaggttttttaaa

SEQ ID NO: 10 - DNA, 3235 bp, synthetic construct
  source 1..3235: mol_type = other DNA
cgttacataacttacggtaaatggcccgcctggctgaccgcccaacgacccccgcccattgacgtcaataatgacgtatgttcccatagtaacgccaatagggactttccattgacgtcaatgggtggagtatttacggtaaactgcccacttggcagtacatcaagtgtatcatatgccaagtacgccccctattgacgtcaatgacggtaaatggcccgcctggcattatgcccagtacatgaccttatgggactttcctacttggcagtacatctacgtattagtcatcgctattaccatggtcgaggtgagccccacgttctgcttcactctccccatctcccccccctccccacccccaattttgtatttatttattttttaattattttgtgcagcgatgggggcggggggggggggggggcgcgcgccaggcggggcggggcggggcgaggggcggggcggggcgaggcggagaggtgcggcggcagccaatcagagcggcgcgctccgaaagtttccttttatggcgaggcggcggcggcggcggccctataaaaagcgaagcgcgcggcgggcgggagtcgctgcgacgctgccttcgccccgtgccccgctccgccgccgcctcgcgccgcccgccccggctctgactgaccgcgttactcccacaggtgagcgggcgggacggcccttctcctccgggctgtaattagctgagcaagaggtaagggtttaagggatggttggttggtggggtattaatgtttaattacctggagcacctgcctgaaatcactttttttcaggttggaccggtgccaccatggacgccatgaagaggggcctgtgttgtgtgctgctgctgtgcggcgccgtgtttgtgagcccccaggtgcagctggtgcagtccggcgctgaggtcatgaagcccggcagctccgtgaaggtgtcctgcaaggcctccggctacacctttagctggtactggctggagtgggtgaggcaggcccctggccacggactggagtggatgggcgagatcgaccctggcacattcactacaaactacaacgagaagttcaaggccagggtgaccttcacagccgatacaagcacctccacagcctacatggagctgagcagcctgaggtccgaggacaccgccgtgtactactgtgccagattttcccacttcagcggctccaactacgactactttgattactggggccagggcacactggtgaccgtgagcagcgcctccaccaagggcccttccgtgttccctctggcccctagctccaagtccacctccggcggcaccgccgctctgggatgtctggtgaaggactacttccccgagcctgtgaccgtgtcctggaactccggcgccctgacatccggcgtgcacaccttccccgccgtgctgcagagctccggcctgtactccctgagcagcgtggtgacagtgccttccagctccctgggcacacagacctacatctgcaacgtgaaccacaagccttccaataccaaggtggacaagaaggtggagcccaagagctgtgataagacccacacctgtcccccttgccctgcccccgagctgctgggaggaccatccgtgttcctgttccctcctaagcctaaggacaccctgatgatctccaggacccccgaggtgacctgcgtggtggtggacgtgtcccacgaggaccctgaggtgaagttcaactggtacgtggatggcgtggaggtgcacaacgccaagacaaagcctagggaggagcagtacaatagcacatacagagtggtgagcgtgctgaccgtgctgcaccaggactggctgaatggcaaggagtacaagtgtaaggtgagcaataaggccctgcccgcccccatcgagaagacaatctccaaggccaagggccagcctagagagccccaggtgtacacactgcccccctccagagacgagctgacaaagaaccaggtgtccctgacatgtctggtgaaaggcttttaccccagcgatatcgccgtggagtgggagagcaatggccagcccgagaataattacaagaccacccctcccgtgctggactccgatggcagctttttcctgtacagcaagctgaccgtggacaagagcagatggcagcagggcaacgtgttctcctgctccgtgatgcacgaggccctgcacaaccactacacccagaagtccctgtccctgtcccctggcaagaggaagagaagggcccccgtgaagcagaccctgaacttcgatctgctgaagctggccggcgatgtggagtccaatcccggccctatggacatgagggtgcccgcccagctgctgggcctgctgctgctgtggctgagcggcgctagatgcgagatcgtgatgacacagtcccccgccaccctgtccgtgagcccaggagagagggccacactgagctgcagggcctcccagagcatcggcaccaatatccactggtaccagcagaagcccggccaggcccctaggctgctgatctactacgcctccgagtccatcagcggcatccccgccagattcagcggcagcggcagcggaaccgagtttaccctgacaatctcctccctgcagtccgaggacttcgccgtgtactattgtcagcagagctggtcctggcccaccacctttggcggcggcacaaaggtggagatcaagaggacagtggccgcccctagcgtgtttatcttcccccccagcgacgagcagctgaagtccggcaccgccagcgtggtgtgtctgctgaacaacttttaccctagggaggccaaggtgcagtggaaggtggataatgccctgcagagcggcaattcccaggagtccgtgacagagcaggatagcaaggacagcacatactccctgtccagcaccctgacactgtccaaggccgactacgagaagcacaaggtgtacgcctgcgaggtgacacaccagggcctgtcctcccctgtgacaaagagcttcaacagaggcgagtgctaggtcgacgtttatttgtgaaatttgtgatgctattgctttatttgtaaccatctagctttatttgtgaaatttgtgatgctattgctttatttgtaaccattataagctgcaataaacaagttaacaacaacaattgcattcattttatgtttcaggttcagggggagatgtgggaggttttttaaa

SEQ ID NO: 11 - DNA, 141 bp, synthetic construct
  source 1..141: mol_type = other DNA
aggaacccctagtgatggagttggccactccctctctgcgcgctcgctcgctcactgaggccgggcgaccaaaggtcgcccgacgcccgggctttgcccgggcggcctcagtgagcgagcgagcgcgcagctgcctgcagg

SEQ ID NO: 12 - DNA, 141 bp, synthetic construct
  source 1..141: mol_type = other DNA
cctgcaggcagctgcgcgctcgctcgctcactgaggccgcccgggcaaagcccgggcgtcgggcgacctttggtcgcccggcctcagtgagcgagcgagcgcgcagagagggagtggccaactccatcactaggggttcct

SEQ ID NO: 13 - DNA, 3898 bp, synthetic construct
  source 1..3898: mol_type = other DNA
acatgtgagcaaaaggccagcaaaaggccaggaaccgtaaaaaggccgcgttgctggcgtttttccataggctccgcccccctgacgagcatcacaaaaatcgacgctcaagtcagaggtggcgaaacccgacaggactataaagataccaggcgtttccccctggaagctccctcgtgcgctctcctgttccgaccctgccgcttaccggatacctgtccgcctttctcccttcgggaagcgtggcgctttctcatagctcacgctgtaggtatctcagttcggtgtaggtcgttcgctccaagctgggctgtgtgcacgaaccccccgttcagcccgaccgctgcgccttatccggtaactatcgtcttgagtccaacccggtaagacacgacttatcgccactggcagcagccactggtaacaggattagcagagcgaggtatgtaggcggtgctacagagttcttgaagtggtggcctaactacggctacactagaaggacagtatttggtatctgcgctctgctgaagccagttaccttcggaaaaagagttggtagctcttgatccggcaaacaaaccaccgctggtagcggtggtttttttgtttgcaagcagcagattacgcgcagaaaaaaaggatctcaagaagatcctttgatcttttctacggggtctgacgctcagtggaacgaaaactcacgttaagggattttggtcatgagattatcaaaaaggatcttcacctagatccttttaaattaaaaatgaagttttaaatcaatctaaagtatatatgagtaaacttggtctgacagttaccaatgcttaatcagtgaggcacctatctcagcgatctgtctatttcgttcatccatagttgcctgactccccgtcgtgtagataactacgatacgggagggcttaccatctggccccagtgctgcaatgataccgcgagacccacgctcaccggctccagatttatcagcaataaaccagccagccggaagggccgagcgcagaagtggtcctgcaactttatccgcctccatccagtctattaattgttgccgggaagctagagtaagtagttcgccagttaatagtttgcgcaacgttgttgccattgctacaggcatcgtggtgtcacgctcgtcgtttggtatggcttcattcagctccggttcccaacgatcaaggcgagttacatgatcccccatgttgtgcaaaaaagcggttagctccttcggtcctccgatcgttgtcagaagtaagttggccgcagtgttatcactcatggttatggcagcactgcataattctcttactgtcatgccatccgtaagatgcttttctgtgactggtgagtactcaaccaagtcattctgagaatagtgtatgcggcgaccgagttgctcttgcccggcgtcaatacgggataataccgcgccacatagcagaactttaaaagtgctcatcattggaaaacgttcttcggggcgaaaactctcaaggatcttaccgctgttgagatccagttcgatgtaacccactcgtgcacccaactgatcttcagcatcttttactttcaccagcgtttctgggtgagcaaaaacaggaaggcaaaatgccgcaaaaaagggaataagggcgacacggaaatgttgaatactcatactcttcctttttcaatattattgaagcatttatcagggttattgtctcatgagcggatacatatttgaatgtatttagaaaaataaacaaataggggttccgcgcacatttccccgaaaagtgccacctgacgtctaagaaaccattattatcatgacattaacctataaaaataggcgtatcacgaggccctttcgtctcgcgcgtttcggtgatgacggtgaaaacctctgacacatgcagctcccggagacggtcacagcttgtctgtaagcggatgccgggagcagacaagcccgtcagggcgcgtcagcgggtgttggcgggtgtcggggctggcttaactatgcggcatcagagcagattgtactgagagtgcaccataaaattgtaaacgttaatattttgttaaaattcgcgttaaatttttgttaaatcagctcattttttaaccaataggccgaaatcggcaaaatcccttataaatcaaaagaatagcccgagatagggttgagtgttgttccagtttggaacaagagtccactattaaagaacgtggactccaacgtcaaagggcgaaaaaccgtctatcagggcgatggcccactacgtgaaccatcacccaaatcaagttttttggggtcgaggtgccgtaaagcactaaatcggaaccctaaagggagcccccgatttagagcttgacggggaaagccggcgaacgtggcgagaaaggaagggaagaaagcgaaaggagcgggcgctagggcgctggcaagtgtagcggtcacgctgcgcgtaaccaccacacccgccgcgcttaatgcgccgctacagggcgcgtactatggttgctttgacgtatgcggtgtgaaataccgcacagatgcgtaaggagaaaataccgcatcaggcgcccctgcaggcagctgcgcgctcgctcgctcactgaggccgcccgggcaaagcccgggcgtcgggcgacctttggtcgcccggcctcagtgagcgagcgagcgcgcagagagggagtggccaactccatcactaggggttcctacgcgtcgttacataacttacggtaaatggcccgcctggctgaccgcccaacgacccccgcccattgacgtcaataatgacgtatgttcccatagtaacgccaatagggactttccattgacgtcaatgggtggagtatttacggtaaactgcccacttggcagtacatcaagtgtatcatatgccaagtacgccccctattgacgtcaatgacggtaaatggcccgcctggcattatgcccagtacatgaccttatgggactttcctacttggcagtacatctacgtattagtcatcgctattaccatggtcgaggtgagccccacgttctgcttcactctccccatctcccccccctccccacccccaattttgtatttatttattttttaattattttgtgcagcgatgggggcggggggggggggggggcgcgcgccaggcggggcggggcggggcgaggggcggggcggggcgaggcggagaggtgcggcggcagccaatcagagcggcgcgctccgaaagtttccttttatggcgaggcggcggcggcggcggccctataaaaagcgaagcgcgcggcgggcgggagtcgctgcgacgctgccttcgccccgtgccccgctccgccgccgcctcgcgccgcccgccccggctctgactgaccgcgttactcccacaggtgagcgggcgggacggcccttctcctccgggctgtaattagctgagcaagaggtaagggtttaagggatggttggttggtggggtattaatgtttaattacctggagcacctgcctgaaatcactttttttcaggttggaccggtgccaccggtcgacgtttatttgtgaaatttgtgatgctattgctttatttgtaaccatctagctttatttgtgaaatttgtgatgctattgctttatttgtaaccattataagctgcaataaacaagttaacaacaacaattgcattcattttatgtttcaggttcagggggagatgtgggaggttttttaaagtttaaacaggaacccctagtgatggagttggccactccctctctgcgcgctcgctcgctcactgaggccgggcgaccaaaggtcgcccgacgcccgggcggcctcagtgagcgagcgagcgcgcagctgcctgcagg

SEQ ID NO: 14 - DNA, 6128 bp, synthetic construct
  source 1..6128: mol_type = other DNA
acatgtgagcaaaaggccagcaaaaggccaggaaccgtaaaaaggccgcgttgctggcgtttttccataggctccgcccccctgacgagcatcacaaaaatcgacgctcaagtcagaggtggcgaaacccgacaggactataaagataccaggcgtttccccctggaagctccctcgtgcgctctcctgttccgaccctgccgcttaccggatacctgtccgcctttctcccttcgggaagcgtggcgctttctcatagctcacgctgtaggtatctcagttcggtgtaggtcgttcgctccaagctgggctgtgtgcacgaaccccccgttcagcccgaccgctgcgccttatccggtaactatcgtcttgagtccaacccggtaagacacgacttatcgccactggcagcagccactggtaacaggattagcagagcgaggtatgtaggcggtgctacagagttcttgaagtggtggcctaactacggctacactagaaggacagtatttggtatctgcgctctgctgaagccagttaccttcggaaaaagagttggtagctcttgatccggcaaacaaaccaccgctggtagcggtggtttttttgtttgcaagcagcagattacgcgcagaaaaaaaggatctcaagaagatcctttgatcttttctacggggtctgacgctcagtggaacgaaaactcacgttaagggattttggtcatgagattatcaaaaaggatcttcacctagatccttttaaattaaaaatgaagttttaaatcaatctaaagtatatatgagtaaacttggtctgacagttaccaatgcttaatcagtgaggcacctatctcagcgatctgtctatttcgttcatccatagttgcctgactccccgtcgtgtagataactacgatacgggagggcttaccatctggccccagtgctgcaatgataccgcgagacccacgctcaccggctccagatttatcagcaataaaccagccagccggaagggccgagcgcagaagtggtcctgcaactttatccgcctccatccagtctattaattgttgccgggaagctagagtaagtagttcgccagttaatagtttgcgcaacgttgttgccattgctacaggcatcgtggtgtcacgctcgtcgtttggtatggcttcattcagctccggttcccaacgatcaaggcgagttacatgatcccccatgttgtgcaaaaaagcggttagctccttcggtcctccgatcgttgtcagaagtaagttggccgcagtgttatcactcatggttatggcagcactgcataattctcttactgtcatgccatccgtaagatgcttttctgtgactggtgagtactcaaccaagtcattctgagaatagtgtatgcggcgaccgagttgctcttgcccggcgtcaatacgggataataccgcgccacatagcagaactttaaaagtgctcatcattggaaaacgttcttcggggcgaaaactctcaaggatcttaccgctgttgagatccagttcgatgtaacccactcgtgcacccaactgatcttcagcatcttttactttcaccagcgtttctgggtgagcaaaaacaggaaggcaaaatgccgcaaaaaagggaataagggcgacacggaaatgttgaatactcatactcttcctttttcaatattattgaagcatttatcagggttattgtctcatgagcggatacatatttgaatgtatttagaaaaataaacaaataggggttccgcgcacatttccccgaaaagtgccacctgacgtctaagaaaccattattatcatgacattaacctataaaaataggcgtatcacgaggccctttcgtctcgcgcgtttcggtgatgacggtgaaaacctctgacacatgcagctcccggagacggtcacagcttgtctgtaagcggatgccgggagcagacaagcccgtcagggcgcgtcagcgggtgttggcgggtgtcggggctggcttaactatgcggcatcagagcagattgtactgagagtgcaccataaaattgtaaacgttaatattttgttaaaattcgcgttaaatttttgttaaatcagctcattttttaaccaataggccgaaatcggcaaaatcccttataaatcaaaagaatagcccgagatagggttgagtgttgttccagtttggaacaagagtccactattaaagaacgtggactccaacgtcaaagggcgaaaaaccgtctatcagggcgatggcccactacgtgaaccatcacccaaatcaagttttttggggtcgaggtgccgtaaagcactaaatcggaaccctaaagggagcccccgatttagagcttgacggggaaagccggcgaacgtggcgagaaaggaagggaagaaagcgaaaggagcgggcgctagggcgctggcaagtgtagcggtcacgctgcgcgtaaccaccacacccgccgcgcttaatgcgccgctacagggcgcgtactatggttgctttgacgtatgcggtgtgaaataccgcacagatgcgtaaggagaaaataccgcatcaggcgcccctgcaggcagctgcgcgctcgctcgctcactgaggccgcccgggcaaagcccgggcgtcgggcgacctttggtcgcccggcctcagtgagcgagcgagcgcgcagagagggagtggccaactccatcactaggggttcctacgcgtcgttacataacttacggtaaatggcccgcctggctgaccgcccaacgacccccgcccattgacgtcaataatgacgtatgttcccatagtaacgccaatagggactttccattgacgtcaatgggtggagtatttacggtaaactgcccacttggcagtacatcaagtgtatcatatgccaagtacgccccctattgacgtcaatgacggtaaatggcccgcctggcattatgcccagtacatgaccttatgggactttcctacttggcagtacatctacgtattagtcatcgctattaccatggtcgaggtgagccccacgttctgcttcactctccccatctcccccccctccccacccccaattttgtatttatttattttttaattattttgtgcagcgatgggggcggggggggggggggggcgcgcgccaggcggggcggggcggggcgaggggcggggcggggcgaggcggagaggtgcggcggcagccaatcagagcggcgcgctccgaaagtttccttttatggcgaggcggcggcggcggcggccctataaaaagcgaagcgcgcggcgggcgggagtcgctgcgacgctgccttcgccccgtgccccgctccgccgccgcctcgcgccgcccgccccggctctgactgaccgcgttactcccacaggtgagcgggcgggacggcccttctcctccgggctgtaattagctgagcaagaggtaagggtttaagggatggttggttggtggggtattaatgtttaattacctggagcacctgcctgaaatcactttttttcaggttggaccggtgccaccatggacgccatgaagaggggcctgtgttgtgtgctgctgctgtgcggcgccgtgtttgtgagcccccaggtgcagctggtgcagtccggcgctgaggtcatgaagcccggcagctccgtgaaggtgtcctgcaaggcctccggctacacctttagctggtactggctggagtgggtgaggcaggcccctggccacggactggagtggatgggcgagatcgaccctggcacattcactacaaactacaacgagaagttcaaggccagggtgaccttcacagccgatacaagcacctccacagcctacatggagctgagcagcctgaggtccgaggacaccgccgtgtactactgtgccagattttcccacttcagcggctccaactacgactactttgattactggggccagggcacactggtgaccgtgagcagcgcctccaccaagggcccttccgtgttccctctggcccctagctccaagtccacctccggcggcaccgccgctctgggatgtctggtgaaggactacttccccgagcctgtgaccgtgtcctggaactccggcgccctgacatccggcgtgcacaccttccccgccgtgctgcagagctccggcctgtactccctgagcagcgtggtgacagtgccttccagctccctgggcacacagacctacatctgcaacgtgaaccacaagccttccaataccaaggtggacaagaaggtggagcccaagagctgtgataagacccacacctgtcccccttgccctgcccccgagctgctgggaggaccatccgtgttcctgttccctcctaagcctaaggacaccctgatgatctccaggacccccgaggtgacctgcgtggtggtggacgtgtcccacgaggaccctgaggtgaagttcaactggtacgtggatggcgtggaggtgcacaacgccaagacaaagcctagggaggagcagtacaatagcacatacagagtggtgagcgtgctgaccgtgctgcaccaggactggctgaatggcaaggagtacaagtgtaaggtgagcaataaggccctgcccgcccccatcgagaagacaatctccaaggccaagggccagcctagagagccccaggtgtacacactgcccccctccagagacgagctgacaaagaaccaggtgtccctgacatgtctggtgaaaggcttttaccccagcgatatcgccgtggagtgggagagcaatggccagcccgagaataattacaagaccacccctcccgtgctggactccgatggcagctttttcctgtacagcaagctgaccgtggacaagagcagatggcagcagggcaacgtgttctcctgctccgtgatgcacgaggccctgcacaaccactacacccagaagtccctgtccctgtcccctggcaagaggaagagaagggcccccgtgaagcagaccctgaacttcgatctgctgaagctggccggcgatgtggagtccaatcccggccctatggacatgagggtgcccgcccagctgctgggcctgctgctgctgtggctgagcggcgctagatgcgagatcgtgatgacacagtcccccgccaccctgtccgtgagcccaggagagagggccacactgagctgcagggcctcccagagcatcggcaccaatatccactggtaccagcagaagcccggccaggcccctaggctgctgatctactacgcctccgagtccatcagcggcatccccgccagattcagcggcagcggcagcggaaccgagtttaccctgacaatctcctccctgcagtccgaggacttcgccgtgtactattgtcagcagagctggtcctggcccaccacctttggcggcggcacaaaggtggagatcaagaggacagtggccgcccctagcgtgtttatcttcccccccagcgacgagcagctgaagtccggcaccgccagcgtggtgtgtctgctgaacaacttttaccctagggaggccaaggtgcagtggaaggtggataatgccctgcagagcggcaattcccaggagtccgtgacagagcaggatagcaaggacagcacatactccctgtccagcaccctgacactgtccaaggccgactacgagaagcacaaggtgtacgcctgcgaggtgacacaccagggcctgtcctcccctgtgacaaagagcttcaacagaggcgagtgctaggtcgacgtttatttgtgaaatttgtgatgctattgctttatttgtaaccatctagctttatttgtgaaatttgtgatgctattgctttatttgtaaccattataagctgcaataaacaagttaacaacaacaattgcattcattttatgtttcaggttcagggggagatgtgggaggttttttaaagtttaaacaggaacccctagtgatggagttggccactccctctctgcgcgctcgctcgctcactgaggccgggcgaccaaaggtcgcccgacgcccgggctttgcccgggcggcctcagtgagcgagcgagcgcgcagctgcctgcagg

SEQ ID NO: 15 - DNA, 714 bp, synthetic construct
  source 1..714: mol_type = other DNA
tctaagctagacccttcagattaaaaataactgaggtaagggcctgggtaggggaggtggtgtgagacgctcctgtctctcctctatctgcccatcggccctttggggaggaggaatgtgcccaaggactaaaaaaaggccatggagccagaggggcgagggcaacagacctttcatgggcaaaccttggggccctgctgtctagcatgccccactacgggtctaggctgcccatgtaaggaggcaaggcctggggacacccgagatgcctggttataattaacccagacatgtggctgcccccccccccccaacacctgctgcctctaaaaataaccctgtccctggtggatcccctgcatgcgaagatcttcgaacaaggctgtgggggactgagggcaggctgtaacaggcttgggggccagggcttatacgtgcctgggactcccaaagtattactgttccatgttcccggcgaagggccagctgtcccccgccagctagactcagcacttagtttaggaaccagtgagcaagtcagcccttggggcagcccatacaaggccatggggctgggcaagctgcacgcctgggtccggggtgggcacggtgcccgggcaacgagctgaaagctcatctgctctcaggggcccctccctggggacagcccctcctggctagtcacaccctgtaggctcctctatataacccagg

SEQ ID NO: 16 - DNA, 564 bp, synthetic construct
  source 1..564: mol_type = other DNA
cagccactatgggtctaggctgcccatgtaaggaggcaaggcctggggacacccgagatgcctggttataattaacccagacatgtggctgctccccccccccaacacctgctgcctgagcctcacccccaccccggtgcctgggtcttaggctctgtacaccatggaggagaagctcgctctaaaaataaccctgtccctggtgggctgtgggggactgagggcaggctgtaacaggcttgggggccagggcttatacgtgcctgggactcccaaagtattactgttccatgttcccggcgaagggccagctgtcccccgccagctagactcagcacttagtttaggaaccagtgagcaagtcagcccttggggcagcccatacaaggccatggggctgggcaagctgcacgcctgggtccggggtgggcacggtgcccgggcaacgagctgaaagctcatctgctctcaggggcccctccctggggacagcccctcctggctagtcacaccctgtaggctcctctatataacccaggggcacaggggctgcccccgggtcac

SEQ ID NO: 17 - DNA, 810 bp, synthetic construct
  source 1..810: mol_type = other DNA
gtttaaacaagcttgcatgtctaagctagacccttcagattaaaaataactgaggtaagggcctgggtaggggaggtggtgtgagacgctcctgtctctcctctatctgcccatcggccctttggggaggaggaatgtgcccaaggactaaaaaaaggccatggagccagaggggcgagggcaacagacctttcatgggcaaaccttggggccctgctgtctagcatgccccactacgggtctaggctgcccatgtaaggaggcaaggcctggggacacccgagatgcctggttataattaacccagacatgtggctgcccccccccccccaacacctgctgcctctaaaaataaccctgtccctggtggatcccctgcatgcgaagatcttcgaacaaggctgtgggggactgagggcaggctgtaacaggcttgggggccagggcttatacgtgcctgggactcccaaagtattactgttccatgttcccggcgaagggccagctgtcccccgccagctagactcagcacttagtttaggaaccagtgagcaagtcagcccttggggcagcccatacaaggccatggggctgggcaagctgcacgcctgggtccggggtgggcacggtgcccgggcaacgagctgaaagctcatctgctctcaggggcccctccctggggacagcccctcctggctagtcacaccctgtaggctcctctatataacccaggggcacaggggctgccctcattctaccaccacctccacagcacagacagacactcaggagccagccagcggcgcgccc

SEQ ID NO: 18 - DNA, 477 bp, synthetic construct
  source 1..477: mol_type = other DNA
gggggaggctgctggtgaatattaaccaaggtcaccccagttatcggaggagcaaacaggggctaagtccactcttgcatctaaaatgagagacaaaaaatctataaaaatggaaaacatgcatagaaatatgtgagggaggaaaaaattacccccaagaatgttagtgcacgcagtcacacagggagaagactatttttgttttgttttgattgttttgttttgttttggttgttttgttttggtgacctaactggtcaaatgacctattaagaatatttcatagaacgaatgttccgatgctctaatctctctagacaaggttcatatttgtatgggttacttattctctctttgttgactaagtcaataatcagaatcagcaggtttgcagtcagattggcagggataagcagcctagctcaggagaagtgagtataaaagccccaggctgggagcagccatcacagaagtcca

SEQ ID NO: 19 - protein, 18 aa, synthetic construct
MKWVTFISLLFLFSSAYS

SEQ ID NO: 20 - protein, 19 aa, synthetic construct
MDWTWRVFCLLAVTPGAHP

SEQ ID NO: 21 - protein, 19 aa, synthetic construct
MAWSPLFLTLITHCAGSWA

SEQ ID NO: 22 - protein, 19 aa, synthetic construct
MTRLTVLALLAGLLASSRA

SEQ ID NO: 23 - protein, 20 aa, synthetic construct
MARPLCTLLLLMATLAGALA

SEQ ID NO: 24 - protein, 20 aa, synthetic construct
MYRMQLLSCIALSLALVTNS

SEQ ID NO: 25 - protein, 22 aa, synthetic construct
MDAMKRGLCCVLLLCGAVFVSP

SEQ ID NO: 26 - protein, 22 aa, synthetic construct
MDMRVPAQLLGLLLLWLSGARC

SEQ ID NO: 27 - protein, 19 aa, synthetic construct
MEFGLSWVFLVALFRGVQC

SEQ ID NO: 28 - DNA, 7336 bp, synthetic construct
  source 1..7336: mol_type = other DNA
atgccggggttttacgagattgtgattaaggtccccagcgaccttgacgagcatctgcccggcatttctgacagctttgtgaactgggtggccgagaaggaatgggagttgccgccagattctgacatggatctgaatctgattgagcaggcacccctgaccgtggccgagaagctgcagcgcgactttctgacggaatggcgccgtgtgagtaaggccccggaggctcttttctttgtgcaatttgagaagggagagagctacttccacatgcacgtgctcgtggaaaccaccggggtgaaatccatggttttgggacgtttcctgagtcagattcgcgaaaaactgattcagagaatttaccgcgggatcgagccgactttgccaaactggttcgcggtcacaaagaccagaaatggcgccggaggcgggaacaaggtggtggatgagtgctacatccccaattacttgctccccaaaacccagcctgagctccagtgggcgtggactaatatggaacagtatttaagcgcctgtttgaatctcacggagcgtaaacggttggtggcgcagcatctgacgcacgtgtcgcagacgcaggagcagaacaaagagaatcagaatcccaattctgatgcgccggtgatcagatcaaaaacttcagccaggtacatggagctggtcgggtggctcgtggacaaggggattacctcggagaagcagtggatccaggaggaccaggcctcatacatctccttcaatgcggcctccaactcgcggtcccaaatcaaggctgccttggacaatgcgggaaagattatgagcctgactaaaaccgcccccgactacctggtgggccagcagcccgtggaggacatttccagcaatcggatttataaaattttggaactaaacgggtacgatccccaatatgcggcttccgtctttctgggatgggccacgaaaaagttcggcaagaggaacaccatctggctgtttgggcctgcaactaccgggaagaccaacatcgcggaggccatagcccacactgtgcccttctacgggtgcgtaaactggaccaatgagaactttcccttcaacgactgtgtcgacaagatggtgatctggtgggaggaggggaagatgaccgccaaggtcgtggagtcggccaaagccattctcggaggaagcaaggtgcgcgtggaccagaaatgcaagtcctcggcccagatagacccgactcccgtgatcgtcacctccaacaccaacatgtgcgccgtgattgacgggaactcaacgaccttcgaacaccagcagccgttgcaagaccggatgttcaaatttgaactcacccgccgtctggatcatgactttgggaaggtcaccaagcaggaagtcaaagactttttccggtgggcaaaggatcacgtggttgaggtggagcatgaattctacgtcaaaaagggtggagccaagaaaagacccgcccccagtgacgcagatataagtgagcccaaacgggtgcgcgagtcagttgcgcagccatcgacgtcagacgcggaagcttcgatcaactacgcagacaggtaccaaaacaaatgttctcgtcacgtgggcatgaatctgatgctgtttccctgcagacaatgcgagagaatgaatcagaattcaaatatctgcttcactcacggacagaaagactgtttagagtgctttcccgtgtcagaatctcaacccgtttctgtcgtcaaaaaggcgtatcagaaactgtgctacattcatcatatcatgggaaaggtgccagacgcttgcactgcctgcgatctggtcaatgtggatttggatgactgcatctttgaacaataaatgatttaaatcaggtatggctgccgatggttatcttccagattggctcgaggacaacctctctgagggcattcgcgagtggtgggcgctgaaacctggagccccgaagcccaaagccaaccagcaaaagcaggacgacggccggggtctggtgcttcctggctacaagtacctcggacccttcaacggactcgacaagggggagcccgtcaacgcggcggacgcagcggccctcgagcacgacaaggcctacgaccagcagctgcaggcgggtgacaatccgtacctgcggtataaccacgccgacgccgagtttcaggagcgtctgcaagaagatacgtcttttgggggcaacctcgggcgagcagtcttccaggccaagaagcgggttctcgaacctctcggtctggttgaggaaggcgctaagacggctcctggaaagaagagaccggtagagccatcaccccagcgttctccagactcctctacgggcatcggcaagaaaggccaacagcccgccagaaaaagactcaattttggtcagactggcgactcagagtcagttccagaccctcaacctctcggagaacctccagcagcgccctctggtgtgggacctaatacaatggctgcaggcggtggcgcaccaatggcagacaataacgaaggcgccgacggagtgggtagttcctcgggaaattggcattgcgattccacatggctgggcgacagagtcatcaccaccagcacccgaacctgggccctgcccacctacaacaaccacctctacaagcaaatctccaacgggacatcgggaggagccaccaacgacaacacctacttcggctacagcaccccctgggggtattttgactttaacagattccactgccacttttcaccacgtgactggcagcgactcatcaacaacaactggggattccggcccaagagactcagcttcaagctcttcaacatccaggtcaaggaggtcacgcagaatgaaggcaccaagaccatcgccaataacctcaccagcaccatccaggtgtttacggactcggagtaccagctgccgtacgttctcggctctgcccaccagggctgcctgcctccgttcccggcggacgtgttcatgattccccagtacggctacctaacactcaacaacggtagtcaggccgtgggacgctcctccttctactgcctggaatactttccttcgcagatgctgagaaccggcaacaacttccagtttacttacaccttcgaggacgtgcctttccacagcagctacgcccacagccagagcttggaccggctgatgaatcctctgattgaccagtacctgtactacttgtctcggactcaaacaacaggaggcacggcaaatacgcagactctgggcttcagccaaggtgggcctaatacaatggccaatcaggcaaagaactggctgccaggaccctgttaccgccaacaacgcgtctcaacgacaaccgggcaaaacaacaatagcaactttgcctggactgctgggaccaaataccatctgaatggaagaaattcattggctaatcctggcatcgctatggcaacacacaaagacgacgaggagcgtttttttcccagtaacgggatcctgatttttggcaaacaaaatgctgccagagacaatgcggattacagcgatgtcatgctcaccagcgaggaagaaatcaaaaccactaaccctgtggctacagaggaatacggtatcgtggcagataacttgcagcagcaaaacacggctcctcaaattggaactgtcaacagccagggggccttacccggtatggtctggcagaaccgggacgtgtacctgcagggtcccatctgggccaagattcctcacacggacggcaacttccacccgtctccgctgatgggcggctttggcctgaaacatcctccgcctcagatcctgatcaagaacacgcctgtacctgcggatcctccgaccaccttcaaccagtcaaagctgaactctttcatcacgcaatacagcaccggacaggtcagcgtggaaattgaatgggagctgcagaaggaaaacagcaagcgctggaaccccgagatccagtacacctccaactactacaaatctacaagtgtggactttgctgttaatacagaaggcgtgtactctgaaccccgccccattggcacccgttacctcacccgtaatctgtaattgcctgttaatcaataaaccggttgattcgtttcagttgaactttggtctctgcgaagggcgaattcgtttaaacctgcaggactagaggtcctgtattagaggtcacgtgagtgttttgcgacattttgcgacaccatgtggtcacgctgggtatttaagcccgagtgagcacgcagggtctccattttgaagcgggaggtttgaacgcgcagccgccaagccgaattctgcagatatccatcacactggcggccgctcgactagagcggccgccaccgcggtggagctccagcttttgttccctttagtgagggttaattgcgcgcttggcgtaatcatggtcatagctgtttcctgtgtgaaattgttatccgctcacaattccacacaacatacgagccggaagcataaagtgtaaagcctggggtgcctaatgagtgagctaactcacattaattgcgttgcgctcactgcccgctttccagtcgggaaacctgtcgtgccagctgcattaatgaatcggccaacgcgcggggagaggcggtttgcgtattgggcgctcttccgcttcctcgctcactgactcgctgcgctcggtcgttcggctgcggcgagcggtatcagctcactcaaaggcggtaatacggttatccacagaatcaggggataacgcaggaaagaacatgtgagcaaaaggccagcaaaaggccaggaaccgtaaaaaggccgcgttgctggcgtttttccataggctccgcccccctgacgagcatcacaaaaatcgacgctcaagtcagaggtggcgaaacccgacaggactataaagataccaggcgtttccccctggaagctccctcgtgcgctctcctgttccgaccctgccgcttaccggatacctgtccgcctttctcccttcgggaagcgtggcgctttctcatagctcacgctgtaggtatctcagttcggtgtaggtcgttcgctccaagctgggctgtgtgcacgaaccccccgttcagcccgaccgctgcgccttatccggtaactatcgtcttgagtccaacccggtaagacacgacttatcgccactggcagcagccactggtaacaggattagcagagcgaggtatgtaggcggtgctacagagttcttgaagtggtggcctaactacggctacactagaagaacagtatttggtatctgcgctctgctgaagccagttaccttcggaaaaagagttggtagctcttgatccggcaaacaaaccaccgctggtagcggtggtttttttgtttgcaagcagcagattacgcgcagaaaaaaaggatctcaagaagatcctttgatcttttctacggggtctgacgctcagtggaacgaaaactcacgttaagggattttggtcatgagattatcaaaaaggatcttcacctagatccttttaaattaaaaatgaagttttaaatcaatctaaagtatatatgagtaaacttggtctgacagttaccaatgcttaatcagtgaggcacctatctcagcgatctgtctatttcgttcatccatagttgcctgactccccgtcgtgtagataactacgatacgggagggcttaccatctggccccagtgctgcaatgataccgcgagacccacgctcaccggctccagatttatcagcaataaaccagccagccggaagggccgagcgcagaagtggtcctgcaactttatccgcctccatccagtctattaattgttgccgggaagctagagtaagtagttcgccagttaatagtttgcgcaacgttgttgccattgctacaggcatcgtggtgtcacgctcgtcgtttggtatggcttcattcagctccggttcccaacgatcaaggcgagttacatgatcccccatgttgtgcaaaaaagcggttagctccttcggtcctccgatcgttgtcagaagtaagttggccgcagtgttatcactcatggttatggcagcactgcataattctcttactgtcatgccatccgtaagatgcttttctgtgactggtgagtactcaaccaagtcattctgagaatagtgtatgcggcgaccgagttgctcttgcccggcgtcaatacgggataataccgcgccacatagcagaactttaaaagtgctcatcattggaaaacgttcttcggggcgaaaactctcaaggatcttaccgctgttgagatccagttcgatgtaacccactcgtgcacccaactgatcttcagcatcttttactttcaccagcgtttctgggtgagcaaaaacaggaaggcaaaatgccgcaaaaaagggaataagggcgacacggaaatgttgaatactcatactcttcctttttcaatattattgaagcatttatcagggttattgtctcatgagcggatacatatttgaatgtatttagaaaaataaacaaataggggttccgcgcacatttccccgaaaagtgccacctaaattgtaagcgttaatattttgttaaaattcgcgttaaatttttgttaaatcagctcattttttaaccaataggccgaaatcggcaaaatcccttataaatcaaaagaatagaccgagatagggttgagtgttgttccagtttggaacaagagtccactattaaagaacgtggactccaacgtcaaagggcgaaaaaccgtctatcagggcgatggcccactacgtgaaccatcaccctaatcaagttttttggggtcgaggtgccgtaaagcactaaatcggaaccctaaagggagcccccgatttagagcttgacggggaaagccggcgaacgtggcgagaaaggaagggaagaaagcgaaaggagcgggcgctagggcgctggcaagtgtagcggtcacgctgcgcgtaaccaccacacccgccgcgcttaatgcgccgctacagggcgcgtcccattcgccattcaggctgcgcaactgttgggaagggcgatcggtgcgggcctcttcgctattacgccagctggcgaaagggggatgtgctgcaaggcgattaagttgggtaacgccagggttttcccagtcacgacgttgtaaaacgacggccagtgagcgcgcgtaatacgactcactatagggcgaattgggtaccgggccccccctcgatcgaggtcgacggtatcgggggagctcgcagggtctccattttgaagcgggaggtttgaacgcgcagccgcc

SEQ ID NO: 29 - DNA, 11635 bp, synthetic construct
  source 1..11635: mol_type = other DNA
ggtacccaactccatgcttaacagtccccaggtacagcccaccctgcgtcgcaaccaggaacagctctacagcttcctggagcgccactcgccctacttccgcagccacagtgcgcagattaggagcgccacttctttttgtcacttgaaaaacatgtaaaaataatgtactaggagacactttcaataaaggcaaatgtttttatttgtacactctcgggtgattatttaccccccacccttgccgtctgcgccgtttaaaaatcaaaggggttctgccgcgcatcgctatgcgccactggcagggacacgttgcgatactggtgtttagtgctccacttaaactcaggcacaaccatccgcggcagctcggtgaagttttcactccacaggctgcgcaccatcaccaacgcgtttagcaggtcgggcgccgatatcttgaagtcgcagttggggcctccgccctgcgcgcgcgagttgcgatacacagggttgcagcactggaacactatcagcgccgggtggtgcacgctggccagcacgctcttgtcggagatcagatccgcgtccaggtcctccgcgttgctcagggcgaacggagtcaactttggtagctgccttcccaaaaagggtgcatgcccaggctttgagttgcactcgcaccgtagtggcatcagaaggtgaccgtgcccggtctgggcgttaggatacagcgcctgcatgaaagccttgatctgcttaaaagccacctgagcctttgcgccttcagagaagaacatgccgcaagacttgccggaaaactgattggccggacaggccgcgtcatgcacgcagcaccttgcgtcggtgttggagatctgcaccacatttcggccccaccggttcttcacgatcttggccttgctagactgctccttcagcgcgcgctgcccgttttcgctcgtcacatccatttcaatcacgtgctccttatttatcataatgctcccgtgtagacacttaagctcgccttcgatctcagcgcagcggtgcagccacaacgcgcagcccgtgggctcgtggtgcttgtaggttacctctgcaaacgactgcaggtacgcctgcaggaatcgccccatcatcgtcacaaaggtcttgttgctggtgaaggtcagctgcaacccgcggtgctcctcgtttagccaggtcttgcatacggccgccagagcttccacttggtcaggcagtagcttgaagtttgcctttagatcgttatccacgtggtacttgtccatcaacgcgcgcgcagcctccatgcccttctcccacgcagacacgatcggcaggctcagcgggtttatcaccgtgctttcactttccgcttcactggactcttccttttcctcttgcgtccgcataccccgcgccactgggtcgtcttcattcagccgccgcaccgtgcgcttacctcccttgccgtgcttgattagcaccggtgggttgctgaaacccaccatttgtagcgccacatcttctctttcttcctcgctgtccacgatcacctctggggatggcgggcgctcgggcttgggagaggggcgcttctttttctttttggacgcaatggccaaatccgccgtcgaggtcgatggccgcgggctgggtgtgcgcggcaccagcgcatcttgtgacgagtcttcttcgtcctcggactcgagacgccgcctcagccgcttttttgggggcgcgcggggaggcggcggcgacggcgacggggacgacacgtcctccatggttggtggacgtcgcgccgcaccgcgtccgcgctcgggggtggtttcgcgctgctcctcttcccgactggccatttccttctcctataggcagaaaaagatcatggagtcagtcgagaaggaggacagcctaaccgccccctttgagttcgccaccaccgcctccaccgatgccgccaacgcgcctaccaccttccccgtcgaggcacccccgcttgaggaggaggaagtgattatcgagcaggacccaggttttgtaagcgaagacgacgaggatcgctcagtaccaacagaggataaaaagcaagaccaggacgacgcagaggcaaacgaggaacaagtcgggcggggggaccaaaggcatggcgactacctagatgtgggagacgacgtgctgttgaagcatctgcagcgccagtgcgccattatctgcgacgcgttgcaagagcgcagcgatgtgcccctcgccatagcggatgtcagccttgcctacgaacgccacctgttctcaccgcgcgtaccccccaaacgccaagaaaacggcacatgcgagcccaacccgcgcctcaacttctaccccgtatttgccgtgccagaggtgcttgccacctatcacatctttttccaaaactgcaagatacccctatcctgccgtgccaaccgcagccgagcggacaagcagctggccttgcggcagggcgctgtcatacctgatatcgcctcgctcgacgaagtgccaaaaatctttgagggtcttggacgcgacgagaaacgcgcggcaaacgctctgcaacaagaaaacagcgaaaatgaaagtcactgtggagtgctggtggaacttgagggtgacaacgcgcgcctagccgtgctgaaacgcagcatcgaggtcacccactttgcctacccggcacttaacctaccccccaaggttatgagcacagtcatgagcgagctgatcgtgcgccgtgcacgacccctggagagggatgcaaacttgcaagaacaaaccgaggagggcctacccgcagttggcgatgagcagctggcgcgctggcttgagacgcgcgagcctgccgacttggaggagcgacgcaagctaatgatggccgcagtgcttgttaccgtggagcttgagtgcatgcagcggttctttgctgacccggagatgcagcgcaagctagaggaaacgttgcactacacctttcgccagggctacgtgcgccaggcctgcaaaatttccaacgtggagctctgcaacctggtctcctaccttggaattttgcacgaaaaccgcctcgggcaaaacgtgcttcattccacgctcaagggcgaggcgcgccgcgactacgtccgcgactgcgtttacttatttctgtgctacacctggcaaacggccatgggcgtgtggcagcaatgcctggaggagcgcaacctaaaggagctgcagaagctgctaaagcaaaacttgaaggacctatggacggccttcaacgagcgctccgtggccgcgcacctggcggacattatcttccccgaacgcctgcttaaaaccctgcaacagggtctgccagacttcaccagtcaaagcatgttgcaaaactttaggaactttatcctagagcgttcaggaattctgcccgccacctgctgtgcgcttcctagcgactttgtgcccattaagtaccgtgaatgccctccgccgctttggggtcactgctaccttctgcagctagccaactaccttgcctaccactccgacatcatggaagacgtgagcggtgacggcctactggagtgtcactgtcgctgcaacctatgcaccccgcaccgctccctggtctgcaattcgcaactgcttagcgaaagtcaaattatcggtacctttgagctgcagggtccctcgcctgacgaaaagtccgcggctccggggttgaaactcactccggggctgtggacgtcggcttaccttcgcaaatttgtacctgaggactaccacgcccacgagattaggttctacgaagaccaatcccgcccgccaaatgcggagcttaccgcctgcgtcattacccagggccacatccttggccaattgcaagccatcaacaaagcccgccaagagtttctgctacgaaagggacggggggtttacctggacccccagtccggcgaggagctcaacccaatccccccgccgccgcagccctatcagcagccgcgggcccttgcttcccaggatggcacccaaaaagaagctgcagctgccgccgccgccacccacggacgaggaggaatactgggacagtcaggcagaggaggttttggacgaggaggaggagatgatggaagactgggacagcctagacgaagcttccgaggccgaagaggtgtcagacgaaacaccgtcaccctcggtcgcattcccctcgccggcgccccagaaattggcaaccgttcccagcatcgctacaacctccgctcctcaggcgccgccggcactgcctgttcgccgacccaaccgtagatgggacaccactggaaccagggccggtaagtctaagcagccgccgccgttagcccaagagcaacaacagcgccaaggctaccgctcgtggcgcgggcacaagaacgccatagttgcttgcttgcaagactgtgggggcaacatctccttcgcccgccgctttcttctctaccatcacggcgtggccttcccccgtaacatcctgcattactaccgtcatctctacagcccctactgcaccggcggcagcggcagcggcagcaacagcagcggtcacacagaagcaaaggcgaccggatagcaagactctgacaaagcccaagaaatccacagcggcggcagcagcaggaggaggagcgctgcgtctggcgcccaacgaacccgtatcgacccgcgagcttagaaataggatttttcccactctgtatgctatatttcaacaaagcaggggccaagaacaagagctgaaaataaaaaacaggtctctgcgctccctcacccgcagctgcctgtatcacaaaagcgaagatcagcttcggcgcacgctggaagacgcggaggctctcttcagcaaatactgcgcgctgactcttaaggactagtttcgcgccctttctcaaatttaagcgcgaaaactacgtcatctccagcggccacacccggcgccagcacctgtcgtcagcgccattatgagcaaggaaattcccacgccctacatgtggagttaccagccacaaatgggacttgcggctggagctgcccaagactactcaacccgaataaactacatgagcgcgggaccccacatgatatcccgggtcaacggaatccgcgcccaccgaaaccgaattctcctcgaacaggcggctattaccaccacacctcgtaataaccttaatccccgtagttggcccgctgccctggtgtaccaggaaagtcccgctcccaccactgtggtacttcccagagacgcccaggccgaagttcagatgactaactcaggggcgcagcttgcgggcggctttcgtcacagggtgcggtcgcccgggcgttttagggcggagtaacttgcatgtattgggaattgtagtttttttaaaatgggaagtgacgtatcgtgggaaaacggaagtgaagatttgaggaagttgtgggttttttggctttcgtttctgggcgtaggttcgcgtgcggttttctgggtgttttttgtggactttaaccgttacgtcattttttagtcctatatatactcgctctgtacttggccctttttacactgtgactgattgagctggtgccgtgtcgagtggtgttttttaataggtttttttactggtaaggctgactgttatggctgccgctgtggaagcgctgtatgttgttctggagcgggagggtgctattttgcctaggcaggagggtttttcaggtgtttatgtgtttttctctcctattaattttgttatacctcctatgggggctgtaatgttgtctctacgcctgcgggtatgtattcccccgggctatttcggtcgctttttagcactgaccgatgttaaccaacctgatgtgtttaccgagtcttacattatgactccggacatgaccgaggaactgtcggtggtgctttttaatcacggtgaccagtttttttacggtcacgccggcatggccgtagtccgtcttatgcttataagggttgtttttcctgttgtaagacaggcttctaatgtttaaatgtttttttttttgttattttattttgtgtttaatgcaggaacccgcagacatgtttgagagaaaaatggtgtctttttctgtggtggttccggaacttacctgcctttatctgcatgagcatgactacgatgtgcttgcttttttgcgcgaggctttgcctgattttttgagcagcaccttgcattttatatcgccgcccatgcaacaagcttacataggggctacgctggttagcatagctccgagtatgcgtgtcataatcagtgtgggttcttttgtcatggttcctggcggggaagtggccgcgctggtccgtgcagacctgcacgattatgttcagctggccctgcgaagggacctacgggatcgcggtatttttgttaatgttccgcttttgaatcttatacaggtctgtgaggaacctgaatttttgcaatcatgattcgctgcttgaggctgaaggtggagggcgctctggagcagatttttacaatggccggacttaatattcgggatttgcttagagacatattgataaggtggcgagatgaaaattatttgggcatggttgaaggtgctggaatgtttatagaggagattcaccctgaagggtttagcctttacgtccacttggacgtgagggcagtttgccttttggaagccattgtgcaacatcttacaaatgccattatctgttctttggctgtagagtttgaccacgccaccggaggggagcgcgttcacttaatagatcttcattttgaggttttggataatcttttggaataaaaaaaaaaaaacatggttcttccagctcttcccgctcctcccgtgtgtgactcgcagaacgaatgtgtaggttggctgggtgtggcttattctgcggtggtggatgttatcagggcagcggcgcatgaaggagtttacatagaacccgaagccagggggcgcctggatgctttgagagagtggatatactacaactactacacagagcgagctaagcgacgagaccggagacgcagatctgtttgtcacgcccgcacctggttttgcttcaggaaatatgactacgtccggcgttccatttggcatgacactacgaccaacacgatctcggttgtctcggcgcactccgtacagtagggatcgcctacctccttttgagacagagacccgcgctaccatactggaggatcatccgctgctgcccgaatgtaacactttgacaatgcacaacgtgagttacgtgcgaggtcttccctgcagtgtgggatttacgctgattcaggaatgggttgttccctgggatatggttctgacgcgggaggagcttgtaatcctgaggaagtgtatgcacgtgtgcctgtgttgtgccaacattgatatcatgacgagcatgatgatccatggttacgagtcctgggctctccactgtcattgttccagtcccggttccctgcagtgcatagccggcgggcaggttttggccagctggtttaggatggtggtggatggcgccatgtttaatcagaggtttatatggtaccgggaggtggtgaattacaacatgccaaaagaggtaatgtttatgtccagcgtgtttatgaggggtcgccacttaatctacctgcgcttgtggtatgatggccacgtgggttctgtggtccccgccatgagctttggatacagcgccttgcactgtgggattttgaacaatattgtggtgctgtgctgcagttactgtgctgatttaagtgagatcagggtgcgctgctgtgcccggaggacaaggcgtctcatgctgcgggcggtgcgaatcatcgctgaggagaccactgccatgttgtattcctgcaggacggagcggcggcggcagcagtttattcgcgcgctgctgcagcaccaccgccctatcctgatgcacgattatgactctacccccatgtaggcgtggacttccccttcgccgcccgttgagcaaccgcaagttggacagcagcctgtggctcagcagctggacagcgacatgaacttaagcgagctgcccggggagtttattaatatcactgatgagcgtttggctcgacaggaaaccgtgtggaatataacacctaagaatatgtctgttacccatgatatgatgctttttaaggccagccggggagaaaggactgtgtactctgtgtgttgggagggaggtggcaggttgaatactagggttctgtgagtttgattaaggtacggtgatcaatataagctatgtggtggtggggctatactactgaatgaaaaatgacttgaaattttctgcaattgaaaaataaacacgttgaaacataacatgcaacaggttcacgattctttattcctgggcaatgtaggagaaggtgtaagagttggtagcaaaagtttcagtggtgtattttccactttcccaggaccatgtaaaagacatagagtaagtgcttacctcgctagtttctgtggattcactagaatcgatgtaggatgttgcccctcctgacgcggtaggagaaggggagggtgccctgcatgtctgccgctgctcttgctcttgccgctgctgaggaggggggcgcatctgccgcagcaccggatgcatctgggaaaagcaaaaaaggggctcgtccctgtttccggaggaatttgcaagcggggtcttgcatgacggggaggcaaacccccgttcgccgcagtccggccggcccgagactcgaaccgggggtcctgcgactcaacccttggaaaataaccctccggctacagggagcgagccacttaatgctttcgctttccagcctaaccgcttacgccgcgcgcggccagtggccaaaaaagctagcgcagcagccgccgcgcctggaaggaagccaaaaggagcgctcccccgttgtctgacgtcgcacacctgggttcgacacgcgggcggtaaccgcatggatcacggcggacggccggatccggggttcgaaccccggtcgtccgccatgatacccttgcgaatttatccaccagaccacggaagagtgcccgcttacaggctctccttttgcacggtctagagcgtcaacgactgcgcacgcctcaccggccagagcgtcccgaccatggagcactttttgccgctgcgcaacatctggaaccgcgtccgcgactttccgcgcgcctccaccaccgccgccggcatcacctggatgtccaggtacatctacggattacgtcgacgtttaaaccatatgatcagctcactcaaaggcggtaatacggttatccacagaatcaggggataacgcaggaaagaacatgtgagcaaaaggccagcaaaaggccaggaaccgtaaaaaggccgcgttgctggcgtttttccataggctccgcccccctgacgagcatcacaaaaatcgacgctcaagtcagaggtggcgaaacccgacaggactataaagataccaggcgtttccccctggaagctccctcgtgcgctctcctgttccgaccctgccgcttaccggatacctgtccgcctttctcccttcgggaagcgtggcgctttctcatagctcacgctgtaggtatctcagttcggtgtaggtcgttcgctccaagctgggctgtgtgcacgaaccccccgttcagcccgaccgctgcgccttatccggtaactatcgtcttgagtccaacccggtaagacacgacttatcgccactggcagcagccactggtaacaggattagcagagcgaggtatgtaggcggtgctacagagttcttgaagtggtggcctaactacggctacactagaagaacagtatttggtatctgcgctctgctgaagccagttaccttcggaaaaagagttggtagctcttgatccggcaaacaaaccaccgctggtagcggtggtttttttgtttgcaagcagcagattacgcgcagaaaaaaaggatctcaagaagatcctttgatcttttctacggggtctgacgctcagtggaacgaaaactcacgttaagggattttggtcatgagattatcaaaaaggatcttcacctagatccttttaaattaaaaatgaagttttaaatcaatctaaagtatatatgagtaaacttggtctgacagttaccaatgcttaatcagtgaggcacctatctcagcgatctgtctatttcgttcatccatagttgcctgactccccgtcgtgtagataactacgatacgggagggcttaccatctggccccagtgctgcaatgataccgcgagacccacgctcaccggctccagatttatcagcaataaaccagccagccggaagggccgagcgcagaagtggtcctgcaactttatccgcctccatccagtctattaattgttgccgggaagctagagtaagtagttcgccagttaatagtttgcgcaacgttgttgccattgctacaggcatcgtggtgtcacgctcgtcgtttggtatggcttcattcagctccggttcccaacgatcaaggcgagttacatgatcccccatgttgtgcaaaaaagcggttagctccttcggtcctccgatcgttgtcagaagtaagttggccgcagtgttatcactcatggttatggcagcactgcataattctcttactgtcatgccatccgtaagatgcttttctgtgactggtgagtactcaaccaagtcattctgagaatagtgtatgcggcgaccgagttgctcttgcccggcgtcaatacgggataataccgcgccacatagcagaactttaaaagtgctcatcattggaaaacgttcttcggggcgaaaactctcaaggatcttaccgctgttgagatccagttcgatgtaacccactcgtgcacccaactgatcttcagcatcttttactttcaccagcgtttctgggtgagcaaaaacaggaaggcaaaatgccgcaaaaaagggaataagggcgacacggaaatgttgaatactcatactcttcctttttcaatattattgaagcatttatcagggttattgtctcatgagcggatacatatttgaatgtatttagaaaaataaacaaataggggttccgcgcacatttccccgaaaagtgccacctaaattgtaagcgttaatattttgttaaaattcgcgttaaatttttgttaaatcagctcattttttaaccaataggccgaaatcggcaaaatcccttataaatcaaaagaatagaccgagatagggttgagtgttgttccagtttggaacaagagtccactattaaagaacgtggactccaacgtcaaagggcgaaaaaccgtctatcagggcgatggcccactacgtgaaccatcaccctaatcaagttttttggggtcgaggtgccgtaaagcactaaatcggaaccctaaagggagcccccgatttagagcttgacggggaaagccggcgaacgtggcgagaaaggaagggaagaaagcgaaaggagcgggcgctagggcgctggcaagtgtagcggtcacgctgcgcgtaaccaccacacccgccgcgcttaatgcgccgctacagggcgcgatggatcc

SEQ ID NO: 30 - DNA, 22 bp, synthetic construct
  source 1..22: mol_type = other DNA
ctgttgtgtgactctggtaact

SEQ ID NO: 31 - DNA, 22 bp, synthetic construct
  source 1..22: mol_type = other DNA
aaatctctagcagtggcgcccg

SEQ ID NO: 32 - DNA, 20 bp, synthetic construct
  source 1..20: mol_type = other DNA
ttcgctttcaagtccctgtt

SEQ ID NO: 33 - DNA, 22 bp, synthetic construct
  source 1..22: mol_type = other DNA
gctgtcatctcttgtgggctgt

SEQ ID NO: 34 - DNA, 26 bp, synthetic construct
  source 1..26: mol_type = other DNA
cctgtcatgcccacacaaatctctcc

SEQ ID NO: 35 - DNA, 21 bp, synthetic construct
  source 1..21: mol_type = other DNA
actcatgggagctgctggttc

SEQ ID NO: 36 - protein, 22 aa, synthetic construct
VKQTLNFDLLKLAGDVESNPGP

SEQ ID NO: 37 - protein, 18 aa, synthetic construct
EGRGSLLTCGDVEENPGP

SEQ ID NO: 38 - protein, 20 aa, synthetic construct
QCTNYALLKLAGDVESNPGP

SEQ ID NO: 39 - protein, 19 aa, synthetic construct
ATNFSLLKQAGDVEENPGP